European Patent Application EP 4 534 096 A1, published April 9, 2025. Title: POLYPEPTIDE AND USE THEREOF IN REGULATING BLOOD GLUCOSE LEVEL AND/OR REDUCING FAT. Applicant: Greenyn Biotechnology Co., Ltd. The sequence listing filed with the application follows.

SEQUENCE LISTING (5 sequences)

SEQ ID NO: 1 - protein, 15 aa, synthetic construct
GGGDATRYSTGGGYS

SEQ ID NO: 2 - protein, 9 aa, synthetic construct
INPNEQREV

SEQ ID NO: 3 - protein, 10 aa, synthetic construct
MQIFVKTLTG

SEQ ID NO: 4 - protein, 6 aa, synthetic construct
MQIFVK

SEQ ID NO: 5 - protein, 8 aa, synthetic construct
VATVIQVL